European Patent Application EP 4 549 469 A1, published May 7, 2025. Title: Antibody targeting melanoma cells. Applicant: Eberhard Karls Universität, Medizinische Fakultät. Application EP. The sequence listing filed with the application follows.

SEQUENCE LISTING (144 sequences)

SEQ ID NO: 1 - protein, 15 aa, synthetic construct
ARLGVTTVVHGAMDY

SEQ ID NO: 2 - protein, 9 aa, synthetic construct
QHHYGTPWT

SEQ ID NO: 3 - protein, 5 aa, synthetic construct
ASGAY

SEQ ID NO: 4 - protein, 9 aa, synthetic construct
QHFWGTPYT

SEQ ID NO: 5 - protein, 12 aa, synthetic construct
ARYYDGYYPLAY

SEQ ID NO: 6 - protein, 9 aa, synthetic construct
LQGTHQPYT

SEQ ID NO: 7 - protein, 12 aa, synthetic construct
ARSGGLRWYFDV

SEQ ID NO: 8 - protein, 9 aa, synthetic construct
QHSWEIPFT

SEQ ID NO: 9 - protein, 19 aa, synthetic construct
ARHAKEVYYSNYDYYAMDY

SEQ ID NO: 10 - protein, 8 aa, synthetic construct
LQYDNLYT

SEQ ID NO: 11 - protein, 11 aa, synthetic construct
AREGYYGNEGY

SEQ ID NO: 12 - protein, 9 aa, synthetic construct
QQGNTLPYT

SEQ ID NO: 13 - protein, 11 aa, synthetic construct
TRDYGYDDFGV

SEQ ID NO: 14 - protein, 9 aa, synthetic construct
QQHYSTPYT

SEQ ID NO: 15 - protein, 13 aa, synthetic construct
ARAYYDYAYYFDY

SEQ ID NO: 16 - protein, 9 aa, synthetic construct
LQSDNMPLT

SEQ ID NO: 17 - protein, 8 aa, synthetic construct
ISSGGSYT

SEQ ID NO: 18 - skipped

SEQ ID NO: 19 - protein, 7 aa, synthetic construct
ILPGSGS

SEQ ID NO: 20 - skipped

SEQ ID NO: 21 - protein, 8 aa, synthetic construct
ILPGSGST

SEQ ID NO: 22 - skipped

SEQ ID NO: 23 - protein, 8 aa, synthetic construct
IYPGNGDT

SEQ ID NO: 24 - skipped

SEQ ID NO: 25 - protein, 8 aa, synthetic construct
FYPGSGSI

SEQ ID NO: 26 - skipped

SEQ ID NO: 27 - protein, 7 aa, synthetic construct
ISYDGSN

SEQ ID NO: 28 - skipped

SEQ ID NO: 29 - protein, 8 aa, synthetic construct
IDPETGGT

SEQ ID NO: 30 - skipped

SEQ ID NO: 31 - protein, 8 aa, synthetic construct
IYPGDGDT

SEQ ID NO: 32 - skipped

SEQ ID NO: 33 - protein, 8 aa, synthetic construct
GFTFSSYG

SEQ ID NO: 34 - protein, 6 aa, synthetic construct
ENIYSY

SEQ ID NO: 35 - protein, 8 aa, synthetic construct
GYTFTGYW

SEQ ID NO: 36 - protein, 6 aa, synthetic construct
ENIYSN

SEQ ID NO: 37 - protein, 8 aa, synthetic construct
GYTFTGYW

SEQ ID NO: 38 - protein, 11 aa, synthetic construct
QSLANSYGNTY

SEQ ID NO: 39 - protein, 8 aa, synthetic construct
GYTFTSYN

SEQ ID NO: 40 - protein, 10 aa, synthetic construct
QSVSTSSYSY

SEQ ID NO: 41 - protein, 8 aa, synthetic construct
GYTFTEYT

SEQ ID NO: 42 - protein, 6 aa, synthetic construct
QDINKY

SEQ ID NO: 43 - protein, 9 aa, synthetic construct
GYSITSGYY

SEQ ID NO: 44 - protein, 6 aa, synthetic construct
QDISNY

SEQ ID NO: 45 - protein, 8 aa, synthetic construct
GYIFIDYE

SEQ ID NO: 46 - protein, 6 aa, synthetic construct
QDVNTA

SEQ ID NO: 47 - protein, 8 aa, synthetic construct
GYTFSNYW

SEQ ID NO: 48 - protein, 6 aa, synthetic construct
TDIDDD

SEQ ID NO: 49 - protein, 122 aa, synthetic construct
EVQLVESGGDLVKPGGSLKLSCAASGFTFSSYGMSWVRQTPDKRLEWVATISSGGSYTYYPDSVKGRFTISRDNAKNTLYLQMSSLKSEDTAMYYCARLGVTTVVHGAMDYWGQGTSVTVSS

SEQ ID NO: 50 - protein, 107 aa, synthetic construct
DIQMTQSPASLSASVGETVTITCRASENIYSYLAWYQQKQGKSPQLLVYNAKTLAEGVPSRFSGSGSGTQFSLKINSLQPEDFGSYYCQHHYGTPWTFGGGTKLEIK

SEQ ID NO: 51 - protein, 112 aa, synthetic construct
QVQLQQSGAELMKPGASVKLSCKATGYTFTGYWIEWVKQRPGHGLEWIGEILPGSGSTNYNEKFKGKATFTADTSSNTAYMQLSSLTTEDSAIYYCASGAYWGQGTLVTVSA

SEQ ID NO: 52 - protein, 107 aa, synthetic construct
DIQMTQSPASLSVSVGETVTITCRASENIYSNLAWYQQKQGKSPQLLVYAATNLADGVPSRFSGSGSGTQYSLKINSLQSEDFGSYYCQHFWGTPYTFGGGTKLEIK

SEQ ID NO: 53 - protein, 119 aa, synthetic construct
QVQLQQSGAELMKPGASVKLSCKATGYTFTGYWIEWVKQRPGHGLEWIGEILPGSGSTNYNEKFKGKATFTADTSSNTAYMQLSSLTTEDSAIYYCARYYDGYYPLAYWGQGTLVTVSA

SEQ ID NO: 54 - protein, 112 aa, synthetic construct
DVVVTQTPLSLPVSFGDQVSISCRSSQSLANSYGNTYLSWYLHKPGQSPQLLIYGISNRFSGVPDRFSGSGSGTDFTLKISTIKPEDLGMYYCLQGTHQPYTFGGGTKLEIK

SEQ ID NO: 55 - protein, 119 aa, synthetic construct
QAYLQQSGAELVRPGASVKMSCKASGYTFTSYNMHWVKQTPRQGLEWIGAIYPGNGDTSYNQKFKGKATLTVDKSSSTAYMQLSSLTSEDSAVYFCARSGGLRWYFDVWGTGTTVTVSS

SEQ ID NO: 56 - protein, 111 aa, synthetic construct
DIVLTQSPASLAVSLGQRATISCRASQSVSTSSYSYMHWYQQKPGQPPKLLIKYASNLESGVPARFSGSGSGTDFTLNIHPVEEEDTATYYCQHSWEIPFTFGSGTKLEIK

SEQ ID NO: 57 - protein, 126 aa, synthetic construct
QVQLQQSGAELVKPGASVKLSCKASGYTFTEYTIHWVKQRSGQGLEWIGWFYPGSGSIKYNEKFKDKATLTADKSSSTVYMELSRLTSEDSAVYFCARHAKEVYYSNYDYYAMDYWGQGTSVTVSS

SEQ ID NO: 58 - protein, 106 aa, synthetic construct
DIQMTQSPSSLSASLGGKVTITCKASQDINKYIAWYQHKPGKGPRLLIHYTSTLQPGIPSRFSGSGSGRDYSFSISNLEPEDIATYYCLQYDNLYTFGGGTKLEIK

SEQ ID NO: 59 - protein, 118 aa, synthetic construct
DVQLQESGPGLVKPSQSLSLTCSVTGYSITSGYYWNWIRQFPGNKLEWMGYISYDGSNNYNPSLKNRISITRDTSKNQFFLKLNSVTTEDTATYYCAREGYYGNEGYWGQGTTLTVSS

SEQ ID NO: 60 - protein, 107 aa, synthetic construct
DIQMTQTTSSLSASLGDRVTISCRASQDISNYLNWYQQKPDGTVKLLIYYTSRLHSGVPSRFSGSGSGTDYSLTISNLEQEDIATYFCQQGNTLPYTFGGGTKLEIK

SEQ ID NO: 61 - protein, 118 aa, synthetic construct
QVQLQQSGAELVRPGASVTLSCKAPGYIFIDYEIHWVKQTPVHGLEWIGAIDPETGGTAYNQKFKGKARLTADISSSTAYMDLRSLTSEDSAVYYCTRDYGYDDFGVWGTGTTVTVSS

SEQ ID NO: 62 - protein, 107 aa, synthetic construct
DIVMTQSHKFMSTSVGDRVNITCKASQDVNTAVAWYQQAPGQSPKLLIYSASYRYTGVPDRFTGSGSGTDFTFTISSVKAEDLAVYYCQQHYSTPYTFGGGTKLEIK

SEQ ID NO: 63 - protein, 120 aa, synthetic construct
QVQLQQSGAELVKPGASVKISCKASGYTFSNYWMNWVKQRPGKGLQWIGQIYPGDGDTNYNGKFEGTATLTADKSSSTAYMQLSSLTSEDSAVYFCARAYYDYAYYFDYWGQGTTLTVSS

SEQ ID NO: 64 - protein, 107 aa, synthetic construct
ETTVTQSPASLSVATGEKVTIRCIISTDIDDDMNWYQQKPGEPPKLLISEGNTLRPGVPSRFSSSGYGTDFVFTIENTLSEDVADYYCLQSDNMPLTFGGGTKLEIK

SEQ ID NO: 65 - protein, 25 aa, synthetic construct
EVQLVESGGDLVKPGGSLKLSCAAS

SEQ ID NO: 66 - protein, 17 aa, synthetic construct
MSWVRQTPDKRLEWVAT

SEQ ID NO: 67 - protein, 38 aa, synthetic construct
YYPDSVKGRFTISRDNAKNTLYLQMSSLKSEDTAMYYC

SEQ ID NO: 68 - protein, 11 aa, synthetic construct
WGQGTSVTVSS

SEQ ID NO: 69 - protein, 26 aa, synthetic construct
DIQMTQSPASLSASVGETVTITCRAS

SEQ ID NO: 70 - protein, 17 aa, synthetic construct
LAWYQQKQGKSPQLLVY

SEQ ID NO: 71 - protein, 36 aa, synthetic construct
TLAEGVPSRFSGSGSGTQFSLKINSLQPEDFGSYYC

SEQ ID NO: 72 - protein, 10 aa, synthetic construct
FGGGTKLEIK

SEQ ID NO: 73 - protein, 25 aa, synthetic construct
QVQLQQSGAELMKPGASVKLSCKAT

SEQ ID NO: 74 - protein, 17 aa, synthetic construct
IEWVKQRPGHGLEWIGE

SEQ ID NO: 75 - protein, 38 aa, synthetic construct
NYNEKFKGKATFTADTSSNTAYMQLSSLTTEDSAIYYC

SEQ ID NO: 76 - protein, 11 aa, synthetic construct
WGQGTLVTVSA

SEQ ID NO: 77 - protein, 26 aa, synthetic construct
DIQMTQSPASLSVSVGETVTITCRAS

SEQ ID NO: 78 - protein, 17 aa, synthetic construct
LAWYQQKQGKSPQLLVY

SEQ ID NO: 79 - protein, 36 aa, synthetic construct
NLADGVPSRFSGSGSGTQYSLKINSLQSEDFGSYYC

SEQ ID NO: 80 - protein, 10 aa, synthetic construct
FGGGTKLEIK

SEQ ID NO: 81 - protein, 25 aa, synthetic construct
QVQLQQSGAELMKPGASVKLSCKAT

SEQ ID NO: 82 - protein, 17 aa, synthetic construct
IEWVKQRPGHGLEWIGE

SEQ ID NO: 83 - protein, 38 aa, synthetic construct; identical to SEQ ID NO: 75

SEQ ID NO: 84 - protein, 11 aa, synthetic construct
WGQGTLVTVSA

SEQ ID NO: 85 - protein, 26 aa, synthetic construct
DVVVTQTPLSLPVSFGDQVSISCRSS

SEQ ID NO: 86 - protein, 17 aa, synthetic construct
LSWYLHKPGQSPQLLIY

SEQ ID NO: 87 - protein, 36 aa, synthetic construct
NRFSGVPDRFSGSGSGTDFTLKISTIKPEDLGMYYC

SEQ ID NO: 88 - protein, 10 aa, synthetic construct
FGGGTKLEIK

SEQ ID NO: 89 - protein, 25 aa, synthetic construct [sequence omitted]

SEQ ID NO: 90 - protein, 17 aa, synthetic construct
MHWVKQTPRQGLEWIGA

SEQ ID NO: 91 - protein, 38 aa, synthetic construct [sequence omitted]

SEQ ID NO: 92 - protein, 11 aa, synthetic construct
WGTGTTVTVSS

SEQ ID NO: 93 - protein, 26 aa, synthetic construct
DIVLTQSPASLAVSLGQRATISCRAS

SEQ ID NO: 94 - protein, 17 aa, synthetic construct
MHWYQQKPGQPPKLLIK

SEQ ID NO: 95 - protein, 36 aa, synthetic construct
NLESGVPARFSGSGSGTDFTLNIHPVEEEDTATYYC

SEQ ID NO: 96 - protein, 10 aa, synthetic construct
FGSGTKLEIK

SEQ ID NO: 97 - protein, 25 aa, synthetic construct
QVQLQQSGAELVKPGASVKLSCKAS

SEQ ID NO: 98 - protein, 17 aa, synthetic construct
IHWVKQRSGQGLEWIGW

SEQ ID NO: 99 - protein, 38 aa, synthetic construct
KYNEKFKDKATLTADKSSSTVYMELSRLTSEDSAVYFC

SEQ ID NO: 100 - protein, 11 aa, synthetic construct
WGQGTSVTVSS

SEQ ID NO: 101 - protein, 26 aa, synthetic construct
DIQMTQSPSSLSASLGGKVTITCKAS

SEQ ID NO: 102 - protein, 17 aa, synthetic construct
IAWYQHKPGKGPRLLIH

SEQ ID NO: 103 - protein, 36 aa, synthetic construct
TLQPGIPSRFSGSGSGRDYSFSISNLEPEDIATYYC

SEQ ID NO: 104 - protein, 10 aa, synthetic construct
FGGGTKLEIK

SEQ ID NO: 105 - protein, 25 aa, synthetic construct
DVQLQESGPGLVKPSQSLSLTCSVT

SEQ ID NO: 106 - protein, 17 aa, synthetic construct
WNWIRQFPGNKLEWMGY

SEQ ID NO: 107 - protein, 38 aa, synthetic construct
NYNPSLKNRISITRDTSKNQFFLKLNSVTTEDTATYYC

SEQ ID NO: 108 - protein, 11 aa, synthetic construct
WGQGTTLTVSS

SEQ ID NO: 109 - protein, 26 aa, synthetic construct
DIQMTQTTSSLSASLGDRVTISCRAS

SEQ ID NO: 110 - protein, 17 aa, synthetic construct
LNWYQQKPDGTVKLLIY

SEQ ID NO: 111 - protein, 36 aa, synthetic construct
RLHSGVPSRFSGSGSGTDYSLTISNLEQEDIATYFC

SEQ ID NO: 112 - protein, 10 aa, synthetic construct
FGGGTKLEIK

SEQ ID NO: 113 - protein, 25 aa, synthetic construct
QVQLQQSGAELVRPGASVTLSCKAP

SEQ ID NO: 114 - protein, 17 aa, synthetic construct
IHWVKQTPVHGLEWIGA

SEQ ID NO: 115 - protein, 38 aa, synthetic construct
AYNQKFKGKARLTADISSSTAYMDLRSLTSEDSAVYYC

SEQ ID NO: 116 - protein, 11 aa, synthetic construct
WGTGTTVTVSS

SEQ ID NO: 117 - protein, 26 aa, synthetic construct
DIVMTQSHKFMSTSVGDRVNITCKAS

SEQ ID NO: 118 - protein, 17 aa, synthetic construct
VAWYQQAPGQSPKLLIY

SEQ ID NO: 119 - protein, 36 aa, synthetic construct
YRYTGVPDRFTGSGSGTDFTFTISSVKAEDLAVYYC

SEQ ID NO: 120 - protein, 10 aa, synthetic construct
FGGGTKLEIK

SEQ ID NO: 121 - protein, 25 aa, synthetic construct
QVQLQQSGAELVKPGASVKISCKAS

SEQ ID NO: 122 - protein, 17 aa, synthetic construct
MNWVKQRPGKGLQWIGQ

SEQ ID NO: 123 - protein, 38 aa, synthetic construct
NYNGKFEGTATLTADKSSSTAYMQLSSLTSEDSAVYFC

SEQ ID NO: 124 - protein, 11 aa, synthetic construct
WGQGTTLTVSS

SEQ ID NO: 125 - protein, 26 aa, synthetic construct
ETTVTQSPASLSVATGEKVTIRCIIS

SEQ ID NO: 126 - protein, 17 aa, synthetic construct
MNWYQQKPGEPPKLLIS

SEQ ID NO: 127 - protein, 36 aa, synthetic construct
TLRPGVPSRFSSSGYGTDFVFTIENTLSEDVADYYC

SEQ ID NO: 128 - protein, 10 aa, synthetic construct
FGGGTKLEIK

SEQ ID NO: 129 - DNA, 367 bp, synthetic construct
  source 1..367: mol_type = other DNA
gaggtgcagctggtggagtctgggggagacttagtgaagcctggagggtccctgaaactctcctgtgcagcctctggattcactttcagtagctatggcatgtcttgggttcgccagactccagacaagaggctggagtgggtcgcaaccattagtagtggtggtagttacacctactatccagacagtgtgaaggggcgattcaccatctccagagacaatgccaagaacaccctgtacctgcaaatgagcagtctgaagtctgaggacacagccatgtattactgtgcaagactgggggttactacggtagtacacggtgctatggactactggggtcaaggaacctcagtcaccgtctcctcag

SEQ ID NO: 130 - DNA, 322 bp, synthetic construct
  source 1..322: mol_type = other DNA
gacatccagatgactcagtctccagcctccctatctgcatctgtgggagaaactgtcaccatcacatgtcgagcaagtgagaatatttacagttatttagcatggtatcagcagaaacagggaaaatctcctcagctcctggtctataatgcaaaaaccttagcagaaggtgtgccatcaaggttcagtggcagtggatcaggcacacagttttctctgaagatcaacagcctgcagcctgaagattttgggagttattactgtcaacatcattatggtactccgtggacgttcggtggaggcaccaagctggaaatcaaac

SEQ ID NO: 131 - DNA, 337 bp, synthetic construct
  source 1..337: mol_type = other DNA
caggttcagctgcagcagtctggagctgagctgatgaagcctggggcctcagtgaagctttcctgcaaggctactggctacacattcactggctactggatagagtgggtaaagcagaggcctggacatggccttgagtggattggagagattttacctggaagtggtagtactaactacaatgagaagttcaagggcaaggccacattcactgcagatacatcctccaacacagcctacatgcaactcagcagcctgacaactgaggactctgccatctattactgtgcaagtggtgcttactggggccaagggactctggtcactgtctctgcag

SEQ ID NO: 132 - DNA, 322 bp, synthetic construct
  source 1..322: mol_type = other DNA
gacatccagatgactcagtctccagcctccctatctgtatctgtgggagaaactgtcaccatcacatgtcgagcaagtgagaatatttacagtaatttagcatggtatcagcagaaacagggaaaatctcctcagctcctggtctatgctgcaacaaacttagcagatggtgtgccatcaaggttcagtggcagtggatcaggcacacagtattccctcaagatcaacagcctgcagtctgaagattttgggagttattactgtcaacatttttggggtactccgtacacgttcggaggggggaccaagctggaaataaaac

SEQ ID NO: 133 - DNA, 358 bp, synthetic construct
  source 1..358: mol_type = other DNA
caggttcagctgcagcagtctggagctgagctgatgaagcctggggcctcagtgaagctttcctgcaaggctactggctacacattcactggctactggatagagtgggtaaagcagaggcctggacatggccttgagtggattggagagattttacctggaagtggtagtactaactacaatgagaagttcaagggcaaggccacattcactgcagatacatcctccaacacagcctacatgcaactcagcagcctgacaactgaggactctgccatctattactgtgcaagatactatgatggttactaccctttggcttactggggccaagggactctggtcactgtctctgcag

SEQ ID NO: 134 - DNA, 337 bp, synthetic construct
  source 1..337: mol_type = other DNA
gatgttgtggtgactcaaactccactctccctgcctgtcagctttggagatcaagtttctatctcttgcaggtctagtcagagtcttgcaaacagttatgggaacacctatttgtcttggtacctgcacaagcctggccagtctccacagctcctcatctatgggatttccaacagattttctggggtgccagacaggttcagtggcagtggttcagggacagatttcacactcaagatcagcacaataaagcctgaggacttgggaatgtattactgcttacaaggtacacatcagccgtacacgttcggaggggggaccaagctggaaataaaac

SEQ ID NO: 135 - DNA, 358 bp, synthetic construct
  source 1..358: mol_type = other DNA
caggcttatctacagcagtctggggctgagctggtgaggcctggggcctcagtgaagatgtcctgcaaggcttctggctacacatttaccagttacaatatgcactgggtaaagcagacacctagacagggcctggaatggattggagctatttatccaggaaatggtgatacttcctacaatcagaagttcaagggcaaggccacactgactgtagacaaatcctccagcacagcctacatgcagctcagcagcctgacatctgaagactctgcggtctatttctgtgcaagatcggggggattacgttggtacttcgatgtctggggcacagggaccacggtcaccgtctcctcag

SEQ ID NO: 136 - DNA, 334 bp, synthetic construct
  source 1..334: mol_type = other DNA
gacattgtgctgacacagtctcctgcttccttagctgtatctctggggcagagggccaccatctcatgcagggccagccaaagtgtcagtacatctagctatagttatatgcactggtaccaacagaaaccaggacagccacccaaactcctcatcaagtatgcatccaacctagaatctggggtccctgccaggttcagtggcagtgggtctgggacagacttcaccctcaacatccatcctgtggaggaggaggatactgcaacatattactgtcagcacagttgggagattccattcacgttcggctcggggacaaagttggaaataaaac

SEQ ID NO: 137 - DNA, 379 bp, synthetic construct
  source 1..379: mol_type = other DNA
caggtccagctgcagcagtctggagctgagctggtgaaacccggggcatcagtgaagctgtcctgcaaggcttctggctacaccttcactgagtatactatacactgggtaaagcagaggtctggacagggtcttgagtggattgggtggttttaccctggaagtggtagtataaagtacaatgagaaattcaaggacaaggccacattgactgcggacaaatcctccagcacagtctatatggagcttagtagattgacatctgaagactctgcggtctatttctgtgcaagacacgcgaaggaggtctactatagtaactacgattactatgctatggactactggggtcaaggaacctcagtcaccgtctcctcag

SEQ ID NO: 138 - DNA, 319 bp, synthetic construct
  source 1..319: mol_type = other DNA
gacatccagatgacacagtctccatcctcactgtctgcatctctgggaggcaaagtcaccatcacttgcaaggcaagccaagacattaacaagtatatagcttggtaccaacacaagcctggaaaaggtcctaggctgctcatacattacacatctacattacagccaggcatcccatcaaggttcagtggaagtgggtctgggagagattattccttcagcatcagcaacctggagcctgaagatattgcaacttattattgtctacagtatgataatctgtacacgttcggaggggggaccaagctggaaataaaac

SEQ ID NO: 139 - DNA, 355 bp, synthetic construct
  source 1..355: mol_type = other DNA
gatgtacagcttcaggagtcaggacctggcctcgtgaaaccttctcagtctctgtctctcacctgctctgtcactggctactccatcaccagtggttattactggaactggatccggcagtttccaggaaacaaactggaatggatgggctacataagctacgatggtagcaataactacaacccatctctcaaaaatcgaatctccatcactcgtgacacatctaagaaccagtttttcctgaagttgaattctgtgactactgaggacacagccacatattactgtgcaagagagggctactatggtaacgaaggctactggggccaaggcaccactctcacagtctcctcag

SEQ ID NO: 140 - DNA, 322 bp, synthetic construct
  source 1..322: mol_type = other DNA
gatatccagatgacacagactacatcctccctgtctgcctctctgggagacagagtcaccatcagttgcagggcaagtcaggacattagcaattatttaaactggtatcagcagaaaccagatggaactgttaaactcctgatctactacacatcaagattacactcaggagtcccatcaaggttcagtggcagtgggtctggaacagattattctctcaccattagcaacctggagcaagaagatattgccacttacttttgccaacagggtaatacgcttccgtacacgttcggaggggggaccaagctggaaataaaac

SEQ ID NO: 141 - DNA, 355 bp, synthetic construct
  source 1..355: mol_type = other DNA
caggttcaactgcagcagtctggggctgagctggtgaggcctggggcttcagtgacgctgtcctgcaaggctccgggctacatatttattgactatgaaatacactgggtgaagcagacacctgtgcatggcctggaatggattggagctattgatcctgaaactggaggtactgcctacaatcagaagttcaagggcaaggccagactgactgcagacatatcctccagtacagcctacatggacctccgcagcctgacatctgaggactctgccgtctattactgtacaagagactatggttacgacgactttggtgtctggggcacagggaccacggtcaccgtctcctcag

SEQ ID NO: 142 - DNA, 322 bp, synthetic construct
  source 1..322: mol_type = other DNA
gacattgtgatgacccagtctcacaaattcatgtccacatcagtaggagacagggtcaacatcacctgcaaggccagtcaggatgtgaatactgctgtagcctggtatcaacaggctccaggacaatctcctaaactactgatttactcggcatcctaccggtacactggagtccctgatcgcttcactggcagtggatctgggacggatttcactttcaccatcagcagtgtgaaggctgaagacctggcagtttattactgtcagcaacattatagtactccgtacacgttcggaggggggaccaagctggaaataaaac

SEQ ID NO: 143 - DNA, 361 bp, synthetic construct
  source 1..361: mol_type = other DNA
caggttcagctgcagcagtctggggctgagctggtgaagcctggggcctcagtgaagatttcctgcaaagcttctggctacacattcagtaactactggatgaactgggtgaagcagaggcctggaaagggtcttcaatggattggacagatttatcctggagatggtgatactaactacaacggaaagttcgagggcacggccacactgactgcagacaaatcctccagcacagcctacatgcagctcagcagcctgacctctgaggactctgcggtctatttctgtgcaagagcctactatgattacgcctactactttgactactggggccaaggcaccactctcacagtctcctcag

SEQ ID NO: 144 - DNA, 322 bp, synthetic construct
  source 1..322: mol_type = other DNA
gaaacaactgtgacccagtctccagcgtccctgtccgtggctacaggagaaaaagtcactatcagatgcataatcagcactgatattgatgatgatatgaactggtaccagcagaagccaggggaacctcctaaactccttatttcagaaggcaatactcttcgtcctggagtcccatcccgattctccagcagtggctatggcacagattttgtttttacaattgaaaacacgctctcagaagatgttgcagattactactgtttgcaaagtgataacatgcctctcacgttcggaggggggaccaagctggaaataaaac